European Patent Application EP 4 786 591 A1, published August 5, 2026. Title: Nucleic acid molecule comprising modified polyadenyl sequence and p53 protein coding sequence. Applicant: HANMI PHARM. CO., LTD. The sequence listing filed with the application follows.

SEQUENCE LISTING (15 sequences)

SEQ ID NO: 1 - DNA, 158 bp, Homo sapiens
  source 1..158: mol_type = genomic DNA
gtgtgtggaggacaccctgaaccccccgctttcaaacaagttttcaaattgtttgaggtcaggatttctcaaactgattcctttctttgcatatgagtatttgaaaataaatattttcccagaatataaataaatcatcacatgattattttaactat

SEQ ID NO: 2 - DNA, 142 bp, synthetic construct
  source 1..142: mol_type = other DNA
aaaaaaaaaaaaaaaaaaaaacaaccagctaagacactgccaaaaaaaaaaaaaaaaaaaaaaaaaaaaaaaaaaaaaaaaaaaaaaaaaaaaaaaaaaaaaaaaaaaaaaaaaaaaaaaaaaaaaaaaaaaaaaaaaaaaa

SEQ ID NO: 3 - DNA, 3103 bp, synthetic construct
  source 1..3103: mol_type = other DNA
aagcttctcgaggtgtgtggaggacaccctgaaccccccgctttcaaacaagttttcaaattgtttgaggtcaggatttctcaaactgattcctttctttgcatatgagtatttgaaaataaatattttcccagaatataaataaatcatcacatgattattttaactatgctagcaaaaaaaaaaaaaaaaaaaaacaaccagctaagacactgccaaaaaaaaaaaaaaaaaaaaaaaaaaaaaaaaaaaaaaaaaaaaaaaaaaaaaaaaaaaaaaaaaaaaaaaaaaaaaaaaaaaaaaaaaaaaaaaaaaaaagaagagcgaattcactggccgtcgttttacagttacccaacttaatcgcctcgcctgatgcggtattttctccttacgcatctgtgcggtatttcacaccgcatatggtgcactctcagtacaatctgctctgatgccgcatagttaagccagccccgacacccgccaacacccgctgacgcgccctgacgggcttgtctgctcccggcatccgcttacagacaagctgtgaccgtctccgggagctgcatgtgtcagaggttttcaccgtcatcaccgaaacgcgcgagacgaaagggcctcgtgatacgcctatttttataggttaatgtcatgataataatggtttcttagacgtcaggtggcacttttcggggaaatgtgcgcggaacccctatttgtttatttttctaaatacattcaaatatgtatccgctcatgagacaataaccctgataaatgcttcaataatattgaaaaagtatgagtattcaacatttccgtgtcgcccttattcccttttttgcggcattttgccttcctgtttttgctcacccagaaacgctggtgaaagtaaaagatgctgaagatcagttgggtgcacgagtgggttacatcgaactggatctcaacagcggtaagatccttgagagttttcgccccgaagaacgttttccatgcagctctggcccgtgtctcaaaatctctgatgttacattgcacaagataaaaatatatcatcatgaacaataaaactgtctgcttacataaacagtaatacaaggggtgttatgagccatattcaacgggaaacgtcgaggccgcgattaaattccaacatggatgctgatttatatgggtataaatgggctcgcgataatgtcgggcaatcaggtgcgacaatctatcgcttgtatgggaagcccgatgcgccagagttgtttctgaaacatggcaaaggtagcgttgccaatgatgttacagatgagatggtcagactaaactggctgacggaatttatgcctcttccgaccatcaagcattttatccgtactcctgatgatgcatggttactcaccactgcgatccccggaaaaacagcattccaggtattagaagaatatcctgattcaggtgaaaatattgttgatgcgctggcagtgttcctgcgccggttgcattcgattcctgtttgtaattgtccttttaacagcgatcgcgtatttcgtctcgctcaggcgcaatcacgaatgaataacggtttggttgatgcgagtgattttgatgacgagcgtaatggctggcctgttgaacaagtctggaaagaaatgcataaacttttgccattctcaccggattcagtcgtcactcatggtgatttctcacttgataaccttatttttgacgaggggaaattaataggttgtattgatgttggacgagtcggaatcgcagaccgataccaggatcttgccatcctatggaactgcctcggtgagttttctccttcattacagaaacggctttttcaaaaatatggtattgataatcctgatatgaataaattgcagtttcatttgatgctcgatgagtttttctaatcagaattggttaattggttgtaacattattcagattgggcttgatttaaaacttcatttttaatttaaaaggatctaggtgaagatcctttttgataatctcatgaccaaaatcccttaacgtgagttttcgttccactgagcgtcagaccccgtagaaaagatcaaaggatcttcttgagatcctttttttctgcgcgtaatctgctgcttgcaaacaaaaaaaccaccgctaccagcggtggtttgtttgccggatcaagagctaccaactctttttccgaaggtaactggcttcagcagagcgcagataccaaatactgttcttctagtgtagccgtagttaggccaccacttcaagaactctgtagcaccgcctacatacctcgctctgctaatcctgttaccagtggctgctgccagtggcgataagtcgtgtcttaccgggttggactcaagacgatagttaccggataaggcgcagcggtcgggctgaacggggggttcgtgcacacagcccagcttggagcgaacgacctacaccgaactgagatacctacagcgtgagctatgagaaagcgccacgcttcccgaagggagaaaggcggacaggtatccggtaagcggcagggtcggaacaggagagcgcacgagggagcttccagggggaaacgcctggtatctttatagtcctgtcgggtttcgccacctctgacttgagcgtcgatttttgtgatgctcgtcaggggggcggagcctatggaaaaacgccagcaacgcggcctttttacggttcctggccttttgctggccttttgcgagccttttgctcacatgttctttcctgcgttatcccctgattctgtggataaccgtattaccgcctttgagtgagctgataccgctcgccgcagccgaacgaccgagcgcagcgagtcagtgagcgaggaagcggcccaatacgcaaaccgcctctccccgcgcgttggccgattcattaatgcagctggcacgacaggtttcccgactggaaagcgggcagtgagcgcaacgcaattaatgtgagttagctcactcattaggcaccccaggctttacactttatgcttccggctcgtatgttgtgtggaattgtgagcggataacaatttcacacaggaaacagctatgaccatgattacgcc

SEQ ID NO: 4 - DNA, 3079 bp, synthetic construct
  source 1..3079: mol_type = other DNA
gtgtgtggaggacaccctgaaccccccgctttcaaacaagttttcaaattgtttgaggtcaggatttctcaaactgattcctttctttgcatatgagtatttgaaaataaatattttcccagaatataaataaatcatcacatgattattttaactataaaaaaaaaaaaaaaaaaaaacaaccagctaagacactgccaaaaaaaaaaaaaaaaaaaaaaaaaaaaaaaaaaaaaaaaaaaaaaaaaaaaaaaaaaaaaaaaaaaaaaaaaaaaaaaaaaaaaaaaaaaaaaaaaaaaagaagagcactggccgtcgttttacagttacccaacttaatcgcctcgcctgatgcggtattttctccttacgcatctgtgcggtatttcacaccgcatatggtgcactctcagtacaatctgctctgatgccgcatagttaagccagccccgacacccgccaacacccgctgacgcgccctgacgggcttgtctgctcccggcatccgcttacagacaagctgtgaccgtctccgggagctgcatgtgtcagaggttttcaccgtcatcaccgaaacgcgcgagacgaaagggcctcgtgatacgcctatttttataggttaatgtcatgataataatggtttcttagacgtcaggtggcacttttcggggaaatgtgcgcggaacccctatttgtttatttttctaaatacattcaaatatgtatccgctcatgagacaataaccctgataaatgcttcaataatattgaaaaagtatgagtattcaacatttccgtgtcgcccttattcccttttttgcggcattttgccttcctgtttttgctcacccagaaacgctggtgaaagtaaaagatgctgaagatcagttgggtgcacgagtgggttacatcgaactggatctcaacagcggtaagatccttgagagttttcgccccgaagaacgttttccatgcagctctggcccgtgtctcaaaatctctgatgttacattgcacaagataaaaatatatcatcatgaacaataaaactgtctgcttacataaacagtaatacaaggggtgttatgagccatattcaacgggaaacgtcgaggccgcgattaaattccaacatggatgctgatttatatgggtataaatgggctcgcgataatgtcgggcaatcaggtgcgacaatctatcgcttgtatgggaagcccgatgcgccagagttgtttctgaaacatggcaaaggtagcgttgccaatgatgttacagatgagatggtcagactaaactggctgacggaatttatgcctcttccgaccatcaagcattttatccgtactcctgatgatgcatggttactcaccactgcgatccccggaaaaacagcattccaggtattagaagaatatcctgattcaggtgaaaatattgttgatgcgctggcagtgttcctgcgccggttgcattcgattcctgtttgtaattgtccttttaacagcgatcgcgtatttcgtctcgctcaggcgcaatcacgaatgaataacggtttggttgatgcgagtgattttgatgacgagcgtaatggctggcctgttgaacaagtctggaaagaaatgcataaacttttgccattctcaccggattcagtcgtcactcatggtgatttctcacttgataaccttatttttgacgaggggaaattaataggttgtattgatgttggacgagtcggaatcgcagaccgataccaggatcttgccatcctatggaactgcctcggtgagttttctccttcattacagaaacggctttttcaaaaatatggtattgataatcctgatatgaataaattgcagtttcatttgatgctcgatgagtttttctaatcagaattggttaattggttgtaacattattcagattgggcttgatttaaaacttcatttttaatttaaaaggatctaggtgaagatcctttttgataatctcatgaccaaaatcccttaacgtgagttttcgttccactgagcgtcagaccccgtagaaaagatcaaaggatcttcttgagatcctttttttctgcgcgtaatctgctgcttgcaaacaaaaaaaccaccgctaccagcggtggtttgtttgccggatcaagagctaccaactctttttccgaaggtaactggcttcagcagagcgcagataccaaatactgttcttctagtgtagccgtagttaggccaccacttcaagaactctgtagcaccgcctacatacctcgctctgctaatcctgttaccagtggctgctgccagtggcgataagtcgtgtcttaccgggttggactcaagacgatagttaccggataaggcgcagcggtcgggctgaacggggggttcgtgcacacagcccagcttggagcgaacgacctacaccgaactgagatacctacagcgtgagctatgagaaagcgccacgcttcccgaagggagaaaggcggacaggtatccggtaagcggcagggtcggaacaggagagcgcacgagggagcttccagggggaaacgcctggtatctttatagtcctgtcgggtttcgccacctctgacttgagcgtcgatttttgtgatgctcgtcaggggggcggagcctatggaaaaacgccagcaacgcggcctttttacggttcctggccttttgctggccttttgcgagccttttgctcacatgttctttcctgcgttatcccctgattctgtggataaccgtattaccgcctttgagtgagctgataccgctcgccgcagccgaacgaccgagcgcagcgagtcagtgagcgaggaagcggcccaatacgcaaaccgcctctccccgcgcgttggccgattcattaatgcagctggcacgacaggtttcccgactggaaagcgggcagtgagcgcaacgcaattaatgtgagttagctcactcattaggcaccccaggctttacactttatgcttccggctcgtatgttgtgtggaattgtgagcggataacaatttcacacaggaaacagctatgaccatgattacgcc

SEQ ID NO: 5 - DNA, 17 bp, synthetic construct
  source 1..17: mol_type = other DNA
taatacgactcactata

SEQ ID NO: 6 - DNA, 61 bp, synthetic construct
  source 1..61: mol_type = other DNA
agtgctccccatccaactaaactgtccctctgtccgaactaaactgcactgtcccagcacc

SEQ ID NO: 7 - DNA, 1179 bp, Homo sapiens
  source 1..1179: mol_type = genomic DNA
atggaagaacctcagtccgatccgagcgtcgagcctcccctgtcacaggaaactttcagtgacctgtggaaactgctgcccgagaataatgtactttcgcctctgcctagccaagcaatggatgatctgatgctgtctccagatgacatcgaacagtggtttacagaggatccagggcccgatgaggcaccacgaatgccagaggcggccccacctgttgcacccgcacctgcggctccaacacccgcagcccccgcccccgctccaagctggcctctcagtagttccgtgccatcacagaagacctatcaaggcagctacggatttcgcctcggatttctccattcaggcactgccaagtccgtgacttgtacgtacagccccgctctgaacaaaatgttctgtcagttggcgaagacatgtcctgtccagctttgggtagattctacccccccgccggggacacgggtgcgagccatggccatttataaacagtctcagcacatgaccgaggtcgtgcgcaggtgtcctcaccatgaacgatgctccgactccgacggcctggcccccccacagcacctgattcgcgtggaaggcaatcttcgtgtggagtacctcgatgatcggaacaccttcagacatagcgtggttgtgccttatgagccacccgaagttggaagcgactgtaccaccatccattacaactatatgtgcaacagtagctgcatgggtggcatgaatcggcggcctatcttgacaataatcactttagaggactcttccggaaacctgcttggcagaaattcattcgaggtccgtgtctgcgcctgcccgggcagggaccgcagaaccgaagaggagaatttacggaaaaagggggaaccccaccacgaactgccaccgggcagtaccaaaagggctctccctaataacacatcttcatcgccccagccaaagaagaaacccctcgacggagagtactttactctacaaattagggggagagaaagatttgagatgttccgcgaattgaacgaggccctggagttgaaagacgctcaagccggaaaggaaccaggtgggtctagggcccactcaagccatctgaagagtaagaaaggccagtccacttccaggcacaaaaagttaatgttcaagacggagggtcctgactctgac

SEQ ID NO: 8 - RNA, 61 nt, synthetic construct
  source 1..61: mol_type = other RNA
agtgctccccatccaactaaactgtccctctgtccgaactaaactgcactgtcccagcacc

SEQ ID NO: 9 - RNA, 1185 nt, Homo sapiens
  source 1..1185: mol_type = mRNA
atggaagaacctcagtccgatccgagcgtcgagcctcccctgtcacaggaaactttcagtgacctgtggaaactgctgcccgagaataatgtactttcgcctctgcctagccaagcaatggatgatctgatgctgtctccagatgacatcgaacagtggtttacagaggatccagggcccgatgaggcaccacgaatgccagaggcggccccacctgttgcacccgcacctgcggctccaacacccgcagcccccgcccccgctccaagctggcctctcagtagttccgtgccatcacagaagacctatcaaggcagctacggatttcgcctcggatttctccattcaggcactgccaagtccgtgacttgtacgtacagccccgctctgaacaaaatgttctgtcagttggcgaagacatgtcctgtccagctttgggtagattctacccccccgccggggacacgggtgcgagccatggccatttataaacagtctcagcacatgaccgaggtcgtgcgcaggtgtcctcaccatgaacgatgctccgactccgacggcctggcccccccacagcacctgattcgcgtggaaggcaatcttcgtgtggagtacctcgatgatcggaacaccttcagacatagcgtggttgtgccttatgagccacccgaagttggaagcgactgtaccaccatccattacaactatatgtgcaacagtagctgcatgggtggcatgaatcggcggcctatcttgacaataatcactttagaggactcttccggaaacctgcttggcagaaattcattcgaggtccgtgtctgcgcctgcccgggcagggaccgcagaaccgaagaggagaatttacggaaaaagggggaaccccaccacgaactgccaccgggcagtaccaaaagggctctccctaataacacatcttcatcgccccagccaaagaagaaacccctcgacggagagtactttactctacaaattagggggagagaaagatttgagatgttccgcgaattgaacgaggccctggagttgaaagacgctcaagccggaaaggaaccaggtgggtctagggcccactcaagccatctgaagagtaagaaaggccagtccacttccaggcacaaaaagttaatgttcaagacggagggtcctgactctgacctcgag

SEQ ID NO: 10 - RNA, 164 nt, synthetic construct
  source 1..164: mol_type = other RNA
gtgtgtggaggacaccctgaaccccccgctttcaaacaagttttcaaattgtttgaggtcaggatttctcaaactgattcctttctttgcatatgagtatttgaaaataaatattttcccagaatataaataaatcatcacatgattattttaactatgctagc

SEQ ID NO: 11 - RNA, 155 nt, synthetic construct
  source 1..155: mol_type = other RNA
aaaaaaaaaaaaaaaaaaaaacaaccagctaagacactgccaaaaaaaaaaaaaaaaaaaaaaaaaaaaaaaaaaaaaaaaaaaaaaaaaaaaaaaaaaaaaaaaaaaaaaaaaaaaaaaaaaaaaaaaaaaaaaaaaaaaaagaagagcgaatt

SEQ ID NO: 12 - RNA, 1179 nt, Homo sapiens
  source 1..1179: mol_type = mRNA
atggaagaacctcagtccgatccgagcgtcgagcctcccctgtcacaggaaactttcagtgacctgtggaaactgctgcccgagaataatgtactttcgcctctgcctagccaagcaatggatgatctgatgctgtctccagatgacatcgaacagtggtttacagaggatccagggcccgatgaggcaccacgaatgccagaggcggccccacctgttgcacccgcacctgcggctccaacacccgcagcccccgcccccgctccaagctggcctctcagtagttccgtgccatcacagaagacctatcaaggcagctacggatttcgcctcggatttctccattcaggcactgccaagtccgtgacttgtacgtacagccccgctctgaacaaaatgttctgtcagttggcgaagacatgtcctgtccagctttgggtagattctacccccccgccggggacacgggtgcgagccatggccatttataaacagtctcagcacatgaccgaggtcgtgcgcaggtgtcctcaccatgaacgatgctccgactccgacggcctggcccccccacagcacctgattcgcgtggaaggcaatcttcgtgtggagtacctcgatgatcggaacaccttcagacatagcgtggttgtgccttatgagccacccgaagttggaagcgactgtaccaccatccattacaactatatgtgcaacagtagctgcatgggtggcatgaatcggcggcctatcttgacaataatcactttagaggactcttccggaaacctgcttggcagaaattcattcgaggtccgtgtctgcgcctgcccgggcagggaccgcagaaccgaagaggagaatttacggaaaaagggggaaccccaccacgaactgccaccgggcagtaccaaaagggctctccctaataacacatcttcatcgccccagccaaagaagaaacccctcgacggagagtactttactctacaaattagggggagagaaagatttgagatgttccgcgaattgaacgaggccctggagttgaaagacgctcaagccggaaaggaaccaggtgggtctagggcccactcaagccatctgaagagtaagaaaggccagtccacttccaggcacaaaaagttaatgttcaagacggagggtcctgactctgac

SEQ ID NO: 13 - RNA, 158 nt, Homo sapiens
  source 1..158: mol_type = mRNA
gtgtgtggaggacaccctgaaccccccgctttcaaacaagttttcaaattgtttgaggtcaggatttctcaaactgattcctttctttgcatatgagtatttgaaaataaatattttcccagaatataaataaatcatcacatgattattttaactat

SEQ ID NO: 14 - RNA, 142 nt, synthetic construct
  source 1..142: mol_type = other RNA
aaaaaaaaaaaaaaaaaaaaacaaccagctaagacactgccaaaaaaaaaaaaaaaaaaaaaaaaaaaaaaaaaaaaaaaaaaaaaaaaaaaaaaaaaaaaaaaaaaaaaaaaaaaaaaaaaaaaaaaaaaaaaaaaaaaaa

SEQ ID NO: 15 - protein, 393 aa, Homo sapiens [sequence omitted]